European Patent Application EP 4 112 068 A1, published January 4, 2023. Title: COMPOSITIONS OF A NEUREGULIN FOR PREVENTING, TREATING OR DELAYING PRESERVED EJECTION FRACTION CARDIAC FAILURE. Applicant: Zensun (Shanghai) Science & Technology, Co., Ltd. Application Divisional application based on EP15850529.7. The sequence listing filed with the application follows.

SEQUENCE LISTING (1 sequence)

SEQ ID NO: 1 - protein, 61 aa, homo sapiens
SHLVKCAEKEKTFCVNGGECFMVKDLSNPSRYLCKCPNEFTGDRCQNYVMASFYKAEELYQ